European Patent Application EP 4 403 575 A1, published July 24, 2024. Title: 包含PD-L1抗原结合片段的组合物及其用途. Applicant: 江苏康宁杰瑞生物制药有限公司. The sequence listing filed with the application follows.

SEQUENCE LISTING (48 sequences)

SEQ ID NO: 1 - protein, 128 aa, synthetic construct
  REGION 1..128: note = 56VH
QVQLQESGGGLVQPGGSLRLSCAASGKMSSRRCMAWFRQAPGKERERVAKLLTTSGSTYLADSVKGRFTISQNNAKSTVYLQMNSLKPEDTAMYYCAADSFEDPTCTLVTSSGAFQYWGQGTQVTVSS

SEQ ID NO: 2 - protein, 128 aa, synthetic construct
  REGION 1..128: note = Hu56V1VH
QVQLVESGGGLVQPGGSLRLSCAASGKMSSRRCMAWFRQAPGKERERVAKLLTTSGSTYLADSVKGRFTISRDNSKNTVYLQMNSLRAEDTAVYYCAADSFEDPTCTLVTSSGAFQYWGQGTLVTVSS

SEQ ID NO: 3 - protein, 128 aa, synthetic construct
  REGION 1..128: note = Hu56V2VH
QVQLVESGGGLVQPGGSLRLSCAASGFTFSRRCMAWFRQAPGKERERVAKLLTTSGSTYLADSVKGRFTISRDNSKNTVYLQMNSLRAEDTAVYYCAADSFEDPTCTLVTSSGAFQYWGQGTLVTVSS

SEQ ID NO: 4 - protein, 128 aa, synthetic construct
  REGION 1..128: note = Hu56V3VH
QVQLVESGGGLVQPGGSLRLSCAASGKMSSRRCMAWFRQAPGKGLERVAKLLTTSGSTYLADSVKGRFTISRDNSKNTVYLQMNSLRAEDTAVYYCAADSFEDPTCTLVTSSGAFQYWGQGTLVTVSS

SEQ ID NO: 5 - protein, 128 aa, synthetic construct
  REGION 1..128: note = Hu56V4VH
QVQLVESGGGLVQPGGSLRLSCAASGFTFSRRCMAWFRQAPGKGLERVAKLLTTSGSTYLADSVKGRFTISRDNSKNTVYLQMNSLRAEDTAVYYCAADSFEDPTCTLVTSSGAFQYWGQGTLVTVSS

SEQ ID NO: 6 - protein, 128 aa, synthetic construct
  REGION 1..128: note = Hu56V5VH
QVQLVESGGGLVQPGGSLRLSCAASGKMSSRRCMAWFRQAPGKERERVAKLLTTSGSTYLADSVKGRFTISRDNSKNTVYLQMNSLKAEDTAVYYCAADSFEDPTCTLVTSSGAFQYWGQGTLVTVSS

SEQ ID NO: 7 - protein, 232 aa, synthetic construct
  REGION 1..232: note = IgG1-Fc
EPKSCDKTHTCPPCPAPELLGGPSVFLFPPKPKDTLMISRTPEVTCVVVDVSHEDPEVKFNWYVDGVEVHNAKTKPREEQYNSTYRVVSVLTVLHQDWLNGKEYKCKVSNKALPAPIEKTISKAKGQPREPQVYTLPPSRDELTKNQVSLTCLVKGFYPSDIAVEWESNGQPENNYKTTPPVLDSDGSFFLYSKLTVDKSRWQQGNVFSCSVMHEALHNHYTQKSLSLSPGK

SEQ ID NO: 8 - protein, 232 aa, synthetic construct
  REGION 1..232: note = IgG1-Fc-m1
EPKSSDKTHTCPPCPAPELLGGPSVFLFPPKPKDTLMISRTPEVTCVVVAVSHEDPEVKFNWYVDGVEVHNAKTKPREEQYNSTYRVVSVLTVLHQDWLNGKEYKCKVSNKALPAGIEKTISKAKGQPREPQVYTLPPSRDELTKNQVSLTCLVKGFYPSDIAVEWESNGQPENNYKTTPPVLDSDGSFFLYSKLTVDKSRWQQGNVFSCSVMHEALHNHYTQKSLSLSPGK

SEQ ID NO: 9 - protein, 232 aa, synthetic construct
  REGION 1..232: note = IgG1-Fc-m2
EPKSSDKTHTCPPCPAPELLGGPSVFLFPPKPKDTLMISRTPEVTCVVVDVSHEDPEVKFNWYVDGVEVHNAKTKPREEQYASTYRVVSVLTVLHQDWLNGKEYKCKVSNKALPAPIEKTISKAKGQPREPQVYTLPPSRDELTKNQVSLTCLVKGFYPSDIAVEWESNGQPENNYKTTPPVLDSDGSFFLYSKLTVDKSRWQQGNVFSCSVMHEALHNHYTQKSLSLSPGK

SEQ ID NO: 10 - protein, 24 aa, synthetic construct
  REGION 1..24: note = linker 1
GTCCTGGCTGCTCTTCTACAAGGC

SEQ ID NO: 11 - protein, 23 aa, synthetic construct
  REGION 1..23: note = linker 2
GGTACGTGCTGTTGAACTGTTCC

SEQ ID NO: 12 - protein, 29 aa, synthetic construct
  REGION 1..29: note = linker 3
GATGTGCAGCTGCAGGAGTCTGGRGGAGG

SEQ ID NO: 13 - protein, 35 aa, synthetic construct
  REGION 1..35: note = linker 4
GGACTAGTGCGGCCGCTGGAGACGGTGACCTGGGT

SEQ ID NO: 14 - protein, 360 aa, synthetic construct
  REGION 1..360: note = 56-Fc
QVQLQESGGGLVQPGGSLRLSCAASGKMSSRRCMAWFRQAPGKERERVAKLLTTSGSTYLADSVKGRFTISQNNAKSTVYLQMNSLKPEDTAMYYCAADSFEDPTCTLVTSSGAFQYWGQGTQVTVSSEPKSCDKTHTCPPCPAPELLGGPSVFLFPPKPKDTLMISRTPEVTCVVVDVSHEDPEVKFNWYVDGVEVHNAKTKPREEQYNSTYRVVSVLTVLHQDWLNGKEYKCKVSNKALPAPIEKTISKAKGQPREPQVYTLPPSRDELTKNQVSLTCLVKGFYPSDIAVEWESNGQPENNYKTTPPVLDSDGSFFLYSKLTVDKSRWQQGNVFSCSVMHEALHNHYTQKSLSLSPGK

SEQ ID NO: 15 - protein, 360 aa, synthetic construct
  REGION 1..360: note = Hu56V1-Fc
QVQLVESGGGLVQPGGSLRLSCAASGKMSSRRCMAWFRQAPGKERERVAKLLTTSGSTYLADSVKGRFTISRDNSKNTVYLQMNSLRAEDTAVYYCAADSFEDPTCTLVTSSGAFQYWGQGTLVTVSSEPKSCDKTHTCPPCPAPELLGGPSVFLFPPKPKDTLMISRTPEVTCVVVDVSHEDPEVKFNWYVDGVEVHNAKTKPREEQYNSTYRVVSVLTVLHQDWLNGKEYKCKVSNKALPAPIEKTISKAKGQPREPQVYTLPPSRDELTKNQVSLTCLVKGFYPSDIAVEWESNGQPENNYKTTPPVLDSDGSFFLYSKLTVDKSRWQQGNVFSCSVMHEALHNHYTQKSLSLSPGK

SEQ ID NO: 16 - protein, 360 aa, synthetic construct
  REGION 1..360: note = Hu56V2-Fc
QVQLVESGGGLVQPGGSLRLSCAASGFTFSRRCMAWFRQAPGKERERVAKLLTTSGSTYLADSVKGRFTISRDNSKNTVYLQMNSLRAEDTAVYYCAADSFEDPTCTLVTSSGAFQYWGQGTLVTVSSEPKSCDKTHTCPPCPAPELLGGPSVFLFPPKPKDTLMISRTPEVTCVVVDVSHEDPEVKFNWYVDGVEVHNAKTKPREEQYNSTYRVVSVLTVLHQDWLNGKEYKCKVSNKALPAPIEKTISKAKGQPREPQVYTLPPSRDELTKNQVSLTCLVKGFYPSDIAVEWESNGQPENNYKTTPPVLDSDGSFFLYSKLTVDKSRWQQGNVFSCSVMHEALHNHYTQKSLSLSPGK

SEQ ID NO: 17 - protein, 360 aa, synthetic construct
  REGION 1..360: note = Hu56V3-Fc
QVQLVESGGGLVQPGGSLRLSCAASGKMSSRRCMAWFRQAPGKGLERVAKLLTTSGSTYLADSVKGRFTISRDNSKNTVYLQMNSLRAEDTAVYYCAADSFEDPTCTLVTSSGAFQYWGQGTLVTVSSEPKSCDKTHTCPPCPAPELLGGPSVFLFPPKPKDTLMISRTPEVTCVVVDVSHEDPEVKFNWYVDGVEVHNAKTKPREEQYNSTYRVVSVLTVLHQDWLNGKEYKCKVSNKALPAPIEKTISKAKGQPREPQVYTLPPSRDELTKNQVSLTCLVKGFYPSDIAVEWESNGQPENNYKTTPPVLDSDGSFFLYSKLTVDKSRWQQGNVFSCSVMHEALHNHYTQKSLSLSPGK

SEQ ID NO: 18 - protein, 359 aa, synthetic construct
  REGION 1..359: note = Hu56V4-Fc
QVQLVESGGGLVQPGGSLRLSCAASGFTFSRRCMAWFRQAPGKGLERVAKLLTTSGSTYLADSVKGRFISRDNSKNTVYLQMNSLRAEDTAVYYCAADSFEDPTCTLVTSSGAFQYWGQGTLVTVSSEPKSCDKTHTCPPCPAPELLGGPSVFLFPPKPKDTLMISRTPEVTCVVVDVSHEDPEVKFNWYVDGVEVHNAKTKPREEQYNSTYRVVSVLTVLHQDWLNGKEYKCKVSNKALPAPIEKTISKAKGQPREPQVYTLPPSRDELTKNQVSLTCLVKGFYPSDIAVEWESNGQPENNYKTTPPVLDSDGSFFLYSKLTVDKSRWQQGNVFSCSVMHEALHNHYTQKSLSLSPGK

SEQ ID NO: 19 - protein, 360 aa, synthetic construct
  REGION 1..360: note = Hu56V5-Fc
QVQLVESGGGLVQPGGSLRLSCAASGKMSSRRCMAWFRQAPGKERERVAKLLTTSGSTYLADSVKGRFTISRDNSKNTVYLQMNSLKAEDTAVYYCAADSFEDPTCTLVTSSGAFQYWGQGTLVTVSSEPKSCDKTHTCPPCPAPELLGGPSVFLFPPKPKDTLMISRTPEVTCVVVDVSHEDPEVKFNWYVDGVEVHNAKTKPREEQYNSTYRVVSVLTVLHQDWLNGKEYKCKVSNKALPAPIEKTISKAKGQPREPQVYTLPPSRDELTKNQVSLTCLVKGFYPSDIAVEWESNGQPENNYKTTPPVLDSDGSFFLYSKLTVDKSRWQQGNVFSCSVMHEALHNHYTQKSLSLSPGK

SEQ ID NO: 20 - protein, 360 aa, synthetic construct
  REGION 1..360: note = 56-Fc-m1
QVQLQESGGGLVQPGGSLRLSCAASGKMSSRRCMAWFRQAPGKERERVAKLLTTSGSTYLADSVKGRFTISQNNAKSTVYLQMNSLKPEDTAMYYCAADSFEDPTCTLVTSSGAFQYWGQGTQVTVSSEPKSSDKTHTCPPCPAPELLGGPSVFLFPPKPKDTLMISRTPEVTCVVVAVSHEDPEVKFNWYVDGVEVHNAKTKPREEQYNSTYRVVSVLTVLHQDWLNGKEYKCKVSNKALPAGIEKTISKAKGQPREPQVYTLPPSRDELTKNQVSLTCLVKGFYPSDIAVEWESNGQPENNYKTTPPVLDSDGSFFLYSKLTVDKSRWQQGNVFSCSVMHEALHNHYTQKSLSLSPGK

SEQ ID NO: 21 - protein, 360 aa, synthetic construct
  REGION 1..360: note = Hu56V1-Fc-m1
QVQLVESGGGLVQPGGSLRLSCAASGKMSSRRCMAWFRQAPGKERERVAKLLTTSGSTYLADSVKGRFTISRDNSKNTVYLQMNSLRAEDTAVYYCAADSFEDPTCTLVTSSGAFQYWGQGTLVTVSSEPKSSDKTHTCPPCPAPELLGGPSVFLFPPKPKDTLMISRTPEVTCVVVAVSHEDPEVKFNWYVDGVEVHNAKTKPREEQYNSTYRVVSVLTVLHQDWLNGKEYKCKVSNKALPAGIEKTISKAKGQPREPQVYTLPPSRDELTKNQVSLTCLVKGFYPSDIAVEWESNGQPENNYKTTPPVLDSDGSFFLYSKLTVDKSRWQQGNVFSCSVMHEALHNHYTQKSLSLSPGK

SEQ ID NO: 22 - protein, 360 aa, synthetic construct
  REGION 1..360: note = Hu56V2-Fc-m1
QVQLVESGGGLVQPGGSLRLSCAASGFTFSRRCMAWFRQAPGKERERVAKLLTTSGSTYLADSVKGRFTISRDNSKNTVYLQMNSLRAEDTAVYYCAADSFEDPTCTLVTSSGAFQYWGQGTLVTVSSEPKSSDKTHTCPPCPAPELLGGPSVFLFPPKPKDTLMISRTPEVTCVVVAVSHEDPEVKFNWYVDGVEVHNAKTKPREEQYNSTYRVVSVLTVLHQDWLNGKEYKCKVSNKALPAGIEKTISKAKGQPREPQVYTLPPSRDELTKNQVSLTCLVKGFYPSDIAVEWESNGQPENNYKTTPPVLDSDGSFFLYSKLTVDKSRWQQGNVFSCSVMHEALHNHYTQKSLSLSPGK

SEQ ID NO: 23 - protein, 360 aa, synthetic construct
  REGION 1..360: note = Hu56V3-Fc-m1
QVQLVESGGGLVQPGGSLRLSCAASGKMSSRRCMAWFRQAPGKGLERVAKLLTTSGSTYLADSVKGRFTISRDNSKNTVYLQMNSLRAEDTAVYYCAADSFEDPTCTLVTSSGAFQYWGQGTLVTVSSEPKSSDKTHTCPPCPAPELLGGPSVFLFPPKPKDTLMISRTPEVTCVVVAVSHEDPEVKFNWYVDGVEVHNAKTKPREEQYNSTYRVVSVLTVLHQDWLNGKEYKCKVSNKALPAGIEKTISKAKGQPREPQVYTLPPSRDELTKNQVSLTCLVKGFYPSDIAVEWESNGQPENNYKTTPPVLDSDGSFFLYSKLTVDKSRWQQGNVFSCSVMHEALHNHYTQKSLSLSPGK

SEQ ID NO: 24 - protein, 360 aa, synthetic construct
  REGION 1..360: note = Hu56V4-Fc-m1
QVQLVESGGGLVQPGGSLRLSCAASGFTFSRRCMAWFRQAPGKGLERVAKLLTTSGSTYLADSVKGRFTISRDNSKNTVYLQMNSLRAEDTAVYYCAADSFEDPTCTLVTSSGAFQYWGQGTLVTVSSEPKSSDKTHTCPPCPAPELLGGPSVFLFPPKPKDTLMISRTPEVTCVVVAVSHEDPEVKFNWYVDGVEVHNAKTKPREEQYNSTYRVVSVLTVLHQDWLNGKEYKCKVSNKALPAGIEKTISKAKGQPREPQVYTLPPSRDELTKNQVSLTCLVKGFYPSDIAVEWESNGQPENNYKTTPPVLDSDGSFFLYSKLTVDKSRWQQGNVFSCSVMHEALHNHYTQKSLSLSPGK

SEQ ID NO: 25 - protein, 360 aa, synthetic construct
  REGION 1..360: note = Hu56V5-Fc-m1
QVQLVESGGGLVQPGGSLRLSCAASGKMSSRRCMAWFRQAPGKERERVAKLLTTSGSTYLADSVKGRFTISRDNSKNTVYLQMNSLKAEDTAVYYCAADSFEDPTCTLVTSSGAFQYWGQGTLVTVSSEPKSSDKTHTCPPCPAPELLGGPSVFLFPPKPKDTLMISRTPEVTCVVVAVSHEDPEVKFNWYVDGVEVHNAKTKPREEQYNSTYRVVSVLTVLHQDWLNGKEYKCKVSNKALPAGIEKTISKAKGQPREPQVYTLPPSRDELTKNQVSLTCLVKGFYPSDIAVEWESNGQPENNYKTTPPVLDSDGSFFLYSKLTVDKSRWQQGNVFSCSVMHEALHNHYTQKSLSLSPGK

SEQ ID NO: 26 - protein, 360 aa, synthetic construct
  REGION 1..360: note = 56-Fc-m2
QVQLQESGGGLVQPGGSLRLSCAASGKMSSRRCMAWFRQAPGKERERVAKLLTTSGSTYLADSVKGRFTISQNNAKSTVYLQMNSLKPEDTAMYYCAADSFEDPTCTLVTSSGAFQYWGQGTQVTVSSEPKSSDKTHTCPPCPAPELLGGPSVFLFPPKPKDTLMISRTPEVTCVVVDVSHEDPEVKFNWYVDGVEVHNAKTKPREEQYASTYRVVSVLTVLHQDWLNGKEYKCKVSNKALPAPIEKTISKAKGQPREPQVYTLPPSRDELTKNQVSLTCLVKGFYPSDIAVEWESNGQPENNYKTTPPVLDSDGSFFLYSKLTVDKSRWQQGNVFSCSVMHEALHNHYTQKSLSLSPGK

SEQ ID NO: 27 - protein, 360 aa, synthetic construct
  REGION 1..360: note = Hu56V1-Fc-m2
QVQLVESGGGLVQPGGSLRLSCAASGKMSSRRCMAWFRQAPGKERERVAKLLTTSGSTYLADSVKGRFTISRDNSKNTVYLQMNSLRAEDTAVYYCAADSFEDPTCTLVTSSGAFQYWGQGTLVTVSSEPKSSDKTHTCPPCPAPELLGGPSVFLFPPKPKDTLMISRTPEVTCVVVDVSHEDPEVKFNWYVDGVEVHNAKTKPREEQYASTYRVVSVLTVLHQDWLNGKEYKCKVSNKALPAPIEKTISKAKGQPREPQVYTLPPSRDELTKNQVSLTCLVKGFYPSDIAVEWESNGQPENNYKTTPPVLDSDGSFFLYSKLTVDKSRWQQGNVFSCSVMHEALHNHYTQKSLSLSPGK

SEQ ID NO: 28 - protein, 360 aa, synthetic construct
  REGION 1..360: note = Hu56V2-Fc-m2
QVQLVESGGGLVQPGGSLRLSCAASGFTFSRRCMAWFRQAPGKERERVAKLLTTSGSTYLADSVKGRFTISRDNSKNTVYLQMNSLRAEDTAVYYCAADSFEDPTCTLVTSSGAFQYWGQGTLVTVSSEPKSSDKTHTCPPCPAPELLGGPSVFLFPPKPKDTLMISRTPEVTCVVVDVSHEDPEVKFNWYVDGVEVHNAKTKPREEQYASTYRVVSVLTVLHQDWLNGKEYKCKVSNKALPAPIEKTISKAKGQPREPQVYTLPPSRDELTKNQVSLTCLVKGFYPSDIAVEWESNGQPENNYKTTPPVLDSDGSFFLYSKLTVDKSRWQQGNVFSCSVMHEALHNHYTQKSLSLSPGK

SEQ ID NO: 29 - protein, 360 aa, synthetic construct
  REGION 1..360: note = Hu56V3-Fc-m2
QVQLVESGGGLVQPGGSLRLSCAASGKMSSRRCMAWFRQAPGKGLERVAKLLTTSGSTYLADSVKGRFTISRDNSKNTVYLQMNSLRAEDTAVYYCAADSFEDPTCTLVTSSGAFQYWGQGTLVTVSSEPKSSDKTHTCPPCPAPELLGGPSVFLFPPKPKDTLMISRTPEVTCVVVDVSHEDPEVKFNWYVDGVEVHNAKTKPREEQYASTYRVVSVLTVLHQDWLNGKEYKCKVSNKALPAPIEKTISKAKGQPREPQVYTLPPSRDELTKNQVSLTCLVKGFYPSDIAVEWESNGQPENNYKTTPPVLDSDGSFFLYSKLTVDKSRWQQGNVFSCSVMHEALHNHYTQKSLSLSPGK

SEQ ID NO: 30 - protein, 360 aa, synthetic construct
  REGION 1..360: note = Hu56V4-Fc-m2
QVQLVESGGGLVQPGGSLRLSCAASGFTFSRRCMAWFRQAPGKGLERVAKLLTTSGSTYLADSVKGRFTISRDNSKNTVYLQMNSLRAEDTAVYYCAADSFEDPTCTLVTSSGAFQYWGQGTLVTVSSEPKSSDKTHTCPPCPAPELLGGPSVFLFPPKPKDTLMISRTPEVTCVVVDVSHEDPEVKFNWYVDGVEVHNAKTKPREEQYASTYRVVSVLTVLHQDWLNGKEYKCKVSNKALPAPIEKTISKAKGQPREPQVYTLPPSRDELTKNQVSLTCLVKGFYPSDIAVEWESNGQPENNYKTTPPVLDSDGSFFLYSKLTVDKSRWQQGNVFSCSVMHEALHNHYTQKSLSLSPGK

SEQ ID NO: 31 - protein, 360 aa, synthetic construct
  REGION 1..360: note = Hu56V5-Fc-m2
QVQLVESGGGLVQPGGSLRLSCAASGKMSSRRCMAWFRQAPGKERERVAKLLTTSGSTYLADSVKGRFTISRDNSKNTVYLQMNSLKAEDTAVYYCAADSFEDPTCTLVTSSGAFQYWGQGTLVTVSSEPKSSDKTHTCPPCPAPELLGGPSVFLFPPKPKDTLMISRTPEVTCVVVDVSHEDPEVKFNWYVDGVEVHNAKTKPREEQYASTYRVVSVLTVLHQDWLNGKEYKCKVSNKALPAPIEKTISKAKGQPREPQVYTLPPSRDELTKNQVSLTCLVKGFYPSDIAVEWESNGQPENNYKTTPPVLDSDGSFFLYSKLTVDKSRWQQGNVFSCSVMHEALHNHYTQKSLSLSPGK

SEQ ID NO: 32 - protein, 448 aa, synthetic construct
  REGION 1..448: note = Human PDL1-Fc
TVTVPKDLYVVEYGSNMTIECKFPVEKQLDLAALIVYWEMEDKNIIQFVHGEEDLKVQHSSYRQRARLLKDQLSLGNAALQITDVKLQDAGVYRCMISYGGADYKRITVKVNAPYNKINQRILVVDPVTSEHELTCQAEGYPKAEVIWTSSDHQVLSGKTTTTNSKREENLFNVTSTLRINTTTNEIFYCTFRRLDPEENHTAELVIPELPLAHPPNERTDDKTHTCPPCPAPELLGGPSVFLFPPKPKDTLMISRTPEVTCVVVDVSHEDPEVKFNWYVDGVEVHNAKTKPREEQYNSTYRVVSVLTVLHQDWLNGKEYKCKVSNKALPAPIEKTISKAKGQPREPQVYTLPPSRDELTKNQVSLTCLVKGFYPSDIAVEWESNGQPENNYKTTPPVLDSDGSFFLYSKLTVDKSRWQQGNVFSCSVMHEALHNHYTQKSLSLSPGK

SEQ ID NO: 33 - protein, 384 aa, synthetic construct
  REGION 1..384: note = antibody 1
QVQLQESGGGLVQPGGSLRLSCAASGKMSSRRCMAWFRQAPGKERERVAKLLTTSGSTYLADSVKGRFTISQNNAKSTVYLQMNSLKPEDTAMYYCAADSFEDPTCTLVTSSGAFQYWGQGTQVTVSSGTCCTGGCTGCTCTTCTACAAGGCEPKSSDKTHTCPPCPAPELLGGPSVFLFPPKPKDTLMISRTPEVTCVVVAVSHEDPEVKFNWYVDGVEVHNAKTKPREEQYNSTYRVVSVLTVLHQDWLNGKEYKCKVSNKALPAGIEKTISKAKGQPREPQVYTLPPSRDELTKNQVSLTCLVKGFYPSDIAVEWESNGQPENNYKTTPPVLDSDGSFFLYSKLTVDKSRWQQGNVFSCSVMHEALHNHYTQKSLSLSPGK

SEQ ID NO: 34 - protein, 383 aa, synthetic construct
  REGION 1..383: note = antibody 2
QVQLVESGGGLVQPGGSLRLSCAASGKMSSRRCMAWFRQAPGKERERVAKLLTTSGSTYLADSVKGRFTISRDNSKNTVYLQMNSLRAEDTAVYYCAADSFEDPTCTLVTSSGAFQYWGQGTLVTVSSGGTACGTGCTGTTGAACTGTTCCEPKSSDKTHTCPPCPAPELLGGPSVFLFPPKPKDTLMISRTPEVTCVVVAVSHEDPEVKFNWYVDGVEVHNAKTKPREEQYNSTYRVVSVLTVLHQDWLNGKEYKCKVSNKALPAGIEKTISKAKGQPREPQVYTLPPSRDELTKNQVSLTCLVKGFYPSDIAVEWESNGQPENNYKTTPPVLDSDGSFFLYSKLTVDKSRWQQGNVFSCSVMHEALHNHYTQKSLSLSPGK

SEQ ID NO: 35 - protein, 389 aa, synthetic construct
  REGION 1..389: note = antibody 3
QVQLVESGGGLVQPGGSLRLSCAASGFTFSRRCMAWFRQAPGKERERVAKLLTTSGSTYLADSVKGRFTISRDNSKNTVYLQMNSLRAEDTAVYYCAADSFEDPTCTLVTSSGAFQYWGQGTLVTVSSGATGTGCAGCTGCAGGAGTCTGGRGGAGGEPKSCDKTHTCPPCPAPELLGGPSVFLFPPKPKDTLMISRTPEVTCVVVDVSHEDPEVKFNWYVDGVEVHNAKTKPREEQYNSTYRVVSVLTVLHQDWLNGKEYKCKVSNKALPAPIEKTISKAKGQPREPQVYTLPPSRDELTKNQVSLTCLVKGFYPSDIAVEWESNGQPENNYKTTPPVLDSDGSFFLYSKLTVDKSRWQQGNVFSCSVMHEALHNHYTQKSLSLSPGK

SEQ ID NO: 36 - protein, 395 aa, synthetic construct
  REGION 1..395: note = antibody 4antibody 8
QVQLVESGGGLVQPGGSLRLSCAASGKMSSRRCMAWFRQAPGKGLERVAKLLTTSGSTYLADSVKGRFTISRDNSKNTVYLQMNSLRAEDTAVYYCAADSFEDPTCTLVTSSGAFQYWGQGTLVTVSSGGACTAGTGCGGCCGCTGGAGACGGTGACCTGGGTEPKSSDKTHTCPPCPAPELLGGPSVFLFPPKPKDTLMISRTPEVTCVVVDVSHEDPEVKFNWYVDGVEVHNAKTKPREEQYASTYRVVSVLTVLHQDWLNGKEYKCKVSNKALPAPIEKTISKAKGQPREPQVYTLPPSRDELTKNQVSLTCLVKGFYPSDIAVEWESNGQPENNYKTTPPVLDSDGSFFLYSKLTVDKSRWQQGNVFSCSVMHEALHNHYTQKSLSLSPGK

SEQ ID NO: 37 - protein, 384 aa, synthetic construct
  REGION 1..384: note = antibody 5
QVQLVESGGGLVQPGGSLRLSCAASGFTFSRRCMAWFRQAPGKGLERVAKLLTTSGSTYLADSVKGRFTISRDNSKNTVYLQMNSLRAEDTAVYYCAADSFEDPTCTLVTSSGAFQYWGQGTLVTVSSGTCCTGGCTGCTCTTCTACAAGGCEPKSSDKTHTCPPCPAPELLGGPSVFLFPPKPKDTLMISRTPEVTCVVVDVSHEDPEVKFNWYVDGVEVHNAKTKPREEQYASTYRVVSVLTVLHQDWLNGKEYKCKVSNKALPAPIEKTISKAKGQPREPQVYTLPPSRDELTKNQVSLTCLVKGFYPSDIAVEWESNGQPENNYKTTPPVLDSDGSFFLYSKLTVDKSRWQQGNVFSCSVMHEALHNHYTQKSLSLSPGK

SEQ ID NO: 38 - protein, 383 aa, synthetic construct
  REGION 1..383: note = antibody 6
QVQLVESGGGLVQPGGSLRLSCAASGKMSSRRCMAWFRQAPGKERERVAKLLTTSGSTYLADSVKGRFTISRDNSKNTVYLQMNSLKAEDTAVYYCAADSFEDPTCTLVTSSGAFQYWGQGTLVTVSSGGTACGTGCTGTTGAACTGTTCCEPKSCDKTHTCPPCPAPELLGGPSVFLFPPKPKDTLMISRTPEVTCVVVDVSHEDPEVKFNWYVDGVEVHNAKTKPREEQYNSTYRVVSVLTVLHQDWLNGKEYKCKVSNKALPAPIEKTISKAKGQPREPQVYTLPPSRDELTKNQVSLTCLVKGFYPSDIAVEWESNGQPENNYKTTPPVLDSDGSFFLYSKLTVDKSRWQQGNVFSCSVMHEALHNHYTQKSLSLSPGK

SEQ ID NO: 39 - protein, 389 aa, synthetic construct
  REGION 1..389: note = antibody 7
QVQLVESGGGLVQPGGSLRLSCAASGKMSSRRCMAWFRQAPGKERERVAKLLTTSGSTYLADSVKGRFTISRDNSKNTVYLQMNSLRAEDTAVYYCAADSFEDPTCTLVTSSGAFQYWGQGTLVTVSSGATGTGCAGCTGCAGGAGTCTGGRGGAGGEPKSSDKTHTCPPCPAPELLGGPSVFLFPPKPKDTLMISRTPEVTCVVVAVSHEDPEVKFNWYVDGVEVHNAKTKPREEQYNSTYRVVSVLTVLHQDWLNGKEYKCKVSNKALPAGIEKTISKAKGQPREPQVYTLPPSRDELTKNQVSLTCLVKGFYPSDIAVEWESNGQPENNYKTTPPVLDSDGSFFLYSKLTVDKSRWQQGNVFSCSVMHEALHNHYTQKSLSLSPGK

SEQ ID NO: 40 - protein, 389 aa, synthetic construct
  REGION 1..389: note = antibody 9
QVQLVESGGGLVQPGGSLRLSCAASGKMSSRRCMAWFRQAPGKERERVAKLLTTSGSTYLADSVKGRFTISRDNSKNTVYLQMNSLKAEDTAVYYCAADSFEDPTCTLVTSSGAFQYWGQGTLVTVSSGATGTGCAGCTGCAGGAGTCTGGRGGAGGEPKSCDKTHTCPPCPAPELLGGPSVFLFPPKPKDTLMISRTPEVTCVVVDVSHEDPEVKFNWYVDGVEVHNAKTKPREEQYNSTYRVVSVLTVLHQDWLNGKEYKCKVSNKALPAPIEKTISKAKGQPREPQVYTLPPSRDELTKNQVSLTCLVKGFYPSDIAVEWESNGQPENNYKTTPPVLDSDGSFFLYSKLTVDKSRWQQGNVFSCSVMHEALHNHYTQKSLSLSPGK

SEQ ID NO: 41 - protein, 389 aa, synthetic construct
  REGION 1..389: note = antibody 10
QVQLQESGGGLVQPGGSLRLSCAASGKMSSRRCMAWFRQAPGKERERVAKLLTTSGSTYLADSVKGRFTISQNNAKSTVYLQMNSLKPEDTAMYYCAADSFEDPTCTLVTSSGAFQYWGQGTQVTVSSGATGTGCAGCTGCAGGAGTCTGGRGGAGGEPKSCDKTHTCPPCPAPELLGGPSVFLFPPKPKDTLMISRTPEVTCVVVDVSHEDPEVKFNWYVDGVEVHNAKTKPREEQYNSTYRVVSVLTVLHQDWLNGKEYKCKVSNKALPAPIEKTISKAKGQPREPQVYTLPPSRDELTKNQVSLTCLVKGFYPSDIAVEWESNGQPENNYKTTPPVLDSDGSFFLYSKLTVDKSRWQQGNVFSCSVMHEALHNHYTQKSLSLSPGK

SEQ ID NO: 42 - protein, 5 aa, synthetic construct
  REGION 1..5: note = linker 5
GGGGS

SEQ ID NO: 43-44 - skipped (2 entries)

SEQ ID NO: 45 - protein, 5 aa, synthetic construct
  REGION 1..5: note = CDR1-1
RRCMA

SEQ ID NO: 46 - protein, 17 aa, synthetic construct
  REGION 1..17: note = CDR2-1
KLLTTSGSTYLADSVKG

SEQ ID NO: 47 - protein, 19 aa, synthetic construct
  REGION 1..19: note = CDR3-1
DSFEDPTCTLVTSSGAFQY

SEQ ID NO: 48 - protein, 10 aa, synthetic construct
  REGION 1..10: note = CDR1-2
GKMSSRRCMA